European Patent Specification EP 3 742 892 B1, published October 18, 2023. Title: Spinach plants resistant to at least Peronospora farinos races 8, 9, 11, 13 and 16. Applicant: Nunhems B.V. The sequence listing filed with the application follows.

SEQUENCE LISTING (10 sequences)

SEQ ID NO: 1 - DNA, 204 bp, Spinacia turkestanica
aacaraaattccgaatgcttcaacgttagttatcttcattggctgctgctgcktttttggtggggaccacaactgggttcctactatytgrttatttagcatgtaaaccgattgcttcgcraaccaatgaccagaagaaaggacaacracatcaaatttcgggatgtcttgcatgaaaacttcatctgggacatcaaggtgcag

SEQ ID NO: 2 - DNA, 204 bp, Spinacia oleracea
aacaraaattccgaatgcttcaacgttagttatcttcattggctgctgctgcktttttggtggggaccacaactgggttcctactatytgrttatttagcatgtagaccgattgcttcgcraaccaatgaccagaagaaaggacaacracatcaaatttcgggatgtcttgcatgaaaacttcatctgggacatcaaggtgcag

SEQ ID NO: 3 - DNA, 299 bp, Spinacia turkestanica
cggtctcctttaccggaattatcgctctcgaggatcggaaaaatgctcgtattacttagggcttgagctgaatctccatcaccaacaagggcaggcaacgatctcgaaagattattcaaattgtaaaatgaagcataattcgcattattattattcgacattctcaatttatcataattagaccggcgtatgccaccatacccgtgtctaaacccatggatcgaccattgataaccgggtttatgaatcattgaatttgttttgactacccctaggggtgaccttttgcaatatccact

SEQ ID NO: 4 - DNA, 299 bp, Spinacia oleracea
cggtctcctttaccggaattatcgctctcgaggatcggaaaaatgctcgtattacttagggcttgagctgaatctccatcaccaacaagggcaggcaacgatctcgaaagattattcaaattgtaaaatgaagcataattcgcattattattattcgacattctcaatttatcataattagacgggcgtatgccaccatacccgtgtctaaacccatggatcgaccattgataaccgggtttatgaatcattgaatttgttttgactacccctaggggtgaccttttgcaatatccact

SEQ ID NO: 5 - DNA, 148 bp, Spinacia tetrandra
gcaaatagatgtgaaataactttttacatatgcaaatatattggaaatagcgaattatatatataatatggtttacataggtttcgacagagggcttactcgtatttatttgaataatatgtcatatttgacgagaataagaatgact

SEQ ID NO: 6 - DNA, 148 bp, Spinacia tetrandra
gctgctgcatcatagggtgatagttccttcctttttcctttatcattggtagatcgtttggcaaaagcctgtggcaccaatacaacaaaaggttaagataaatttgtttgctatgaccatattctaatcaaaagaacatagcaacata

SEQ ID NO: 7 - DNA, 299 bp, Spinacia oleracea
ggaagaacattagtactagcttaattgaatattccataactttttatttttgcttaattagattgtggtttgaagctatgcaaatagatgtgaaataactttttatttttgcttaattagattgtggtttgaagctatgcaaatagatgtgaaatagcgaatatatattatataatatggtttacatagatttcgacagaggggttactcgtatttgtttgaataatatttcatatttgatgaaaaatagggattacttaatcttaaaatagcatttatgctttactctaagggtgtta

SEQ ID NO: 8 - DNA, 237 bp, Spinacia oleracea
gcaacggcaagctctcgaagggcacgtagggccttagatctgcgaataaggtaagccctgaaggtccactggatcaaagctgctgcatcatagggtgatagttccttcctttttcctttatcattggtagatcttttggcaaaagcctgtatggcaccaatacaacaaaaggttaagataaatttgtttgctatgaccatattctaatcaaaagaacatagcaacatattcaagggg

SEQ ID NO: 9 - DNA, 204 bp, unknown
  Spinachbase sequence of Figure 1
aacagaaattccgaatgcttcaacgttagttatcttcattggctgctgctgcgtttttggtggggaccacaactgggttcctactatctggttatttagcatgtaaaccgattgcttcgcaaaccaatgaccagaagaaaggacaacaacatcaaatttcgggatgtcttgcatgaaaacttcatctgggacatcaaggtgcag

SEQ ID NO: 10 - DNA, 305 bp, unknown
  Spinachbase sequence of Figure 2
cggtctcctttaccggaattatcgctctcgaggatcggaaaaatgctcgtattatttagggtttgagctgaatctccatcaccaataagggcaggcaatgatctcgaaagattattcaaattgtaaaatgaagcataattcgcgttattattattattattcgacattctcaatttatcataattagacgggcgtattccaccatacccgtgtctaaacccatggatcgaccattgataaccgggtttatgaatcattgaatttgttttgactacccctaggggtgaccttttgcaatatccact